European Patent Application EP 4 721 573 A1, published April 8, 2026. Title: COMBINATION OF ENDOLYSISN AND GLUCOSE OXIDASE AND USES THEREOF. Applicant: Consejo Superior de Investigaciones Cientificas (CSIC). The sequence listing filed with the application follows.

SEQUENCE LISTING (3 sequences)

SEQ ID NO: 1 - protein, 316 aa, phage vB_LmoS_188
  source 1..316: note = amino acid sequence of N-acetylmuramoyl-L-alanine amidase of the phage vB_LmoS_188; note (original language) = secuencia de aminoacidos de N-acetilmuramoil-L-alanina amidasa del fago vB_LmoS_188
MSVLQYNYINKNQFSRPGYKLLRVSKIVMHYTANPGASADNHRRYFRDLKERYASAHIFIDDNEAICIIPLNEVAYHANERSCKLTALQASTSYYRGGNANLTSIGIEMCLDKNGNITAATFNRSVDVAAELCKTYDLTASDIIRHYDVTGKNCPAPWVAKPSELTRFRNAVNAKLKGASQNKNRHDGKVVDSAPLLPKMDFKSSPFRMYKSGTEFLVYEHNQYWYKTYINDKLYYMYKSFCDVVAKKDAKGRIPVKIKSAKDLRIPVWDNTRLNSGKIKWYKPGTKLSWYDNKKGYLELWYDKDGWYYTANYFLK

SEQ ID NO: 2 - protein, 308 aa, phage PSU-VKH-LP041
  source 1..308: note = amino acid sequence of N-acetylmuramoyl-L-alanine amidase of the phage PSU-VKH-LP041; note (original language) = secuencia de aminoacidos de la N-acetilmuramoil-L-alanina amidasa del fago PSU-VKH-LP041
MATVNGVPFRQNLVSSSKYSIKAPNTMKAKKITIHNTYNNASSQNETDYCKNNNNEVSFHVAVDDKEAIQVVPFGRNAWHCGDGGNGYGNRNTIGVETCYSKSGGAKYIAAEKNTIKYVAGLCVQQDIIASKDTIKKHQDWSGKYCPHRILDDKRWPAVQQAIIDEYNRITSKNPNRHSGQVVDSAPLLPKTDFKSNPARMYKSGTEFLVYEHNQYWYKTYIDDKLYYMYKSFCDVVAKKDAKGRIKVRIKSAKDLRIPVWNNTKLSSGKIKWYKPGTKLSWYNNKKGYLELWYTNDGWYYTANYFLK

SEQ ID NO: 3 - protein, 583 aa, synthetic construct
  source 1..583: note = amino acid sequence of glucose oxidase; note (original language) = secuencia de aminoacidos de glucosa oxidasa; organism (original language) = construccion sintetica
SNGIEASLLTDPKDVSGRTVDYIIAGGGLTGLTTAARLTENPNISVLVIESGSYESDRGPIIEDLNAYGDIFGSSVDHAYETVELATNNRTALIRSGNGLGGSTLVNGGTWTRPHKAQVDSWETVFGNEGWNWDNVAAYSLQAERARAPNAKQIAAGHYFNASCHGTNGTVHAGPRDTGDDYSPIVKALMSAVEDRGVPTKKDFGCGDPHGVSMFPNTLHEDQVRSDAAREWLLPNYQRPNLQVLTGQYVGKVLLSQNGTTPRAVGVEFGTHKGNTHNVYAEHEVLLAAGSAVSPTILEYSGIGMKSILEPLGIDTVVDLPVGLNLQDQTTATVRSRITSAGAGQGQAAWFATFNETFGDYSEKAHELLNTKLEQWAEEAVARGGFHNTTALLIQYENYRDWIVNHNVAYSELFLDTAGVASFDVWDLLPFTRGYVHILDKDPYLHHFAYDPQYFLNELDLLGQAAATQLARNISNSGAMQTYFAGETIPGDNLAYDADLSAWTEYIPEHFRPNYHGVGTCSMMPKEMGGVVDNAARVYGVQGLRVIDGSIPPMQMSSHVMTVFYAMALKISDAILEDYASMQ